European Patent Specification EP 3 785 718 B1, published March 27, 2024. Title: MEDICINAL COMPOSITION FOR PREVENTING OR TREATING FLAVIVIRUS INFECTIONS AND METHOD FOR TREATING THE SAME. Applicant: LEMONEX INC. The sequence listing filed with the application follows.

SEQUENCE LISTING (6 sequences)

SEQ ID NO: 1 - DNA, 21 bp, Artificial Sequence
  Human GAPDH Forward primer
tcactgccacccagaagactg

SEQ ID NO: 2 - DNA, 19 bp, Artificial Sequence
  Human GAPDH Reverse primer
ggatgaccttgcccacagc

SEQ ID NO: 3 - DNA, 23 bp, Artificial Sequence
  Mouse GAPDH Forward primer
tgacctcaactacatggtctaca

SEQ ID NO: 4 - DNA, 19 bp, Artificial Sequence
  Mouse GAPDH Reverse primer
cttcccattctcggccttg

SEQ ID NO: 5 - DNA, 25 bp, Artificial Sequence
  DV2 NS1 Forward primer
gctccttcaatgacaatgcgctgta

SEQ ID NO: 6 - DNA, 23 bp, Artificial Sequence
  DV2 NS1 Reverse primer
cctgaaaccccttccacgaagtc